European Patent Application EP 4 400 174 A2, published July 17, 2024. Title: IMMUNOREGULATORY MOLECULES AND USES THEREFOR. Applicant: The Francis Crick Institute Limited. The sequence listing filed with the application follows.

SEQUENCE LISTING (6 sequences)

SEQ ID NO: 1 - DNA, 429 bp, Homo sapiens
  source 1..429: mol_type = genomic DNA
atgggacttaagttgaacggcagatatatttcactgatcctcgcggtgcaaatagcgtatctggtgcaggccgtgagagcagcgggcaagtgcgatgcggtcttcaagggcttttcggactgtttgctcaagctgggcgacagcatggccaactacccgcagggcctggacgacaagacgaacatcaagaccgtgtgcacatactgggaggatttccacagctgcacggtcacagcccttacggattgccaggaaggggcgaaagatatgtgggataaactgagaaaagaatccaaaaacctcaacatccaaggcagcttattcgaactctgcggcagcggcaacggggcggcggggtccctgctcccggcgttcccggtgctcctggtgtctctctcggcagctttagcgacctggctttccttctga

SEQ ID NO: 2 - protein, 142 aa, Homo sapiens
MGLKLNGRYISLILAVQIAYLVQAVRAAGKCDAVFKGFSDCLLKLGDSMANYPQGLDDKTNIKTVCTYWEDFHSCTVTALTDCQEGAKDMWDKLRKESKNLNIQGSLFELCGSGNGAAGSLLPAFPVLLVSLSAALATWLSF

SEQ ID NO: 3 - DNA, 348 bp, Homo sapiens
  source 1..348: mol_type = genomic DNA
gcgggcaagtgcgatgcggtcttcaagggcttttcggactgtttgctcaagctgggcgacagcatggccaactacccgcagggcctggacgacaagacgaacatcaagaccgtgtgcacatactgggaggatttccacagctgcacggtcacagcccttacggattgccaggaaggggcgaaagatatgtgggataaactgagaaaagaatccaaaaacctcaacatccaaggcagcttattcgaactctgcggcagcggcaacggggcggcggggtccctgctcccggcgttcccggtgctcctggtgtctctctcggcagctttagcgacctggctttccttctga

SEQ ID NO: 4 - protein, 115 aa, Homo sapiens
AGKCDAVFKGFSDCLLKLGDSMANYPQGLDDKTNIKTVCTYWEDFHSCTVTALTDCQEGAKDMWDKLRKESKNLNIQGSLFELCGSGNGAAGSLLPAFPVLLVSLSAALATWLSF

SEQ ID NO: 5 - DNA, 267 bp, Homo sapiens
  source 1..267: mol_type = genomic DNA
gcgggcaagtgcgatgcggtcttcaagggcttttcggactgtttgctcaagctgggcgacagcatggccaactacccgcagggcctggacgacaagacgaacatcaagaccgtgtgcacatactgggaggatttccacagctgcacggtcacagcccttacggattgccaggaaggggcgaaagatatgtgggataaactgagaaaagaatccaaaaacctcaacatccaaggcagcttattcgaactctgcggcagcggcaacggg

SEQ ID NO: 6 - protein, 89 aa, Homo sapiens
AGKCDAVFKGFSDCLLKLGDSMANYPQGLDDKTNIKTVCTYWEDFHSCTVTALTDCQEGAKDMWDKLRKESKNLNIQGSLFELCGSGNG